European Patent Specification EP 3 188 758 B1, published October 4, 2023. Title: SIRP ALPHA-ANTIBODY FUSION PROTEINS. Applicant: The Board of Trustees of the Leland Stanford Junior University. The sequence listing filed with the application follows.

SEQUENCE LISTING (15 sequences)

SEQ ID NO: 1 - protein, 119 aa, Homo sapiens
EEELQVIQPDKSVLVAAGETATLRCTATSLIPVGPIQWFRGAGPGRELIYNQKEGHFPRVTTVSDLTKRNNMDFSIRIGNITPADAGTYYCVKFRKGSPDDVEFKSGAGTELSVRAKPS

SEQ ID NO: 2 - protein, 5 aa, H. sapiens
GGGGS

SEQ ID NO: 3 - protein, 13 aa, H. sapiens
ASTKGPSVFPLAP

SEQ ID NO: 4 - DNA, 708 bp, H. sapiens
  CDS (1)...(708)
atggattttcaggtgcagattatcagcttcctgctaatcagtgcttcagtcataatgtccagaggacaaattgttctctcccagtctccagcaatcctgtctgcatctccaggggagaaggtcacaatgacttgcagggccagctcaagtgtaagttacatccactggttccagcagaagccaggatcctcccccaaaccctggatttatgccacatccaacctggcttctggagtccctgttcgcttcagtggcagtgggtctgggacttcttactctctcaccatcagcagagtggaggctgaagatgctgccacttattactgccagcagtggactagtaacccacccacgttcggaggggggaccaagctggaaatcaaacgtacggtggcggcgccatctgtcttcatcttcccgccatctgatgagcagttgaaatctggaactgcctctgttgtgtgcctgctgaataacttctatcccagagaggccaaagtacagtggaaggtggataacgccctccaatcgggtaactcccaggagagtgtcacagagcaggacagcaaggacagcacctacagcctcagcagcaccctgacgctgagcaaagcagactacgagaaacacaaagtctacgcctgcgaagtcacccatcagggcctgagctcgcccgtcacaaagagcttcaacaggggagagtgttag

SEQ ID NO: 5 - protein, 235 aa, H. sapiens
MDFQVQIISFLLISASVIMSRGQIVLSQSPAILSASPGEKVTMTCRASSSVSYIHWFQQKPGSSPKPWIYATSNLASGVPVRFSGSGSGTSYSLTISRVEAEDAATYYCQQWTSNPPTFGGGTKLEIKRTVAAPSVFIFPPSDEQLKSGTASVVCLLNNFYPREAKVQWKVDNALQSGNSQESVTEQDSKDSTYSLSSTLTLSKADYEKHKVYACEVTHQGLSSPVTKSFNRGEC

SEQ ID NO: 6 - DNA, 1800 bp, H. sapiens
  CDS (1)...(1800)
atgggttggagcctcatcttgctcttccttgtcgctgttgctacgcgtgtcctgtcccaggtacaactgcagcagcctggggctgagctggtgaagcctggggcctcagtgaagatgtcctgcaaggcttctggctacacatttaccagttacaatatgcactgggtaaaacagacacctggtcggggcctggaatggattggagctatttatcccggaaatggtgatacttcctacaatcagaagttcaaaggcaaggccacattgactgcagacaaatcctccagcacagcctacatgcagctcagcagcctgacatctgaggactctgcggtctattactgtgcaagatcgacttactacggcggtgactggtacttcaatgtctggggcgcagggaccacggtcaccgtctctgcagcgagcaccaagggcccatcggtcttccccctggcaccctcctccaagagcacctctgggggcacagcggccctgggctgcctggtcaaggactacttccccgaaccggtgacggtgtcgtggaactcaggcgccctgaccagcggcgtgcacaccttcccggctgtcctacagtcctcaggactctactccctcagcagcgtggtgaccgtgccctccagcagcttgggcacccagacctacatctgcaacgtgaatcacaagcccagcaacaccaaggtggacaagaaagttgagcccaaatcttgtgacaaaactcacacatgcccaccgtgcccagcacctgaactcctggggggaccgtcagtcttcctcttccccccaaaacccaaggacaccctcatgatctcccggacccctgaggtcacatgcgtggtggtggacgtgagccacgaagaccctgaggtcaagttcaactggtacgtggacggcgtggaggtgcataatgccaagacaaagccgcgggaggagcagtacaacagcacgtaccgtgtggtcagcgtcctcaccgtcctgcaccaggactggctgaatggcaaggagtacaagtgcaaggtctccaacaaagccctcccagcccccatcgagaaaaccatctccaaagccaaagggcagccccgagaaccacaggtgtacaccctgcccccatcccgggatgagctgaccaagaaccaggtcagcctgacctgcctggtcaaaggcttctatcccagcgacatcgccgtggagtgggagagcaatgggcagccggagaacaactacaagaccacgcctcccgtgctggactccgacggctccttcttcctctacagcaagctcaccgtggacaagagcaggtggcagcaggggaacgtcttctcatgctccgtgatgcatgaggctctgcacaaccactacacgcagaagagcctctccctgtctccgggtaaaggtggcggtggctcgggcggtggtgggtcggaggaggagctgcaggtgattcagcctgacaagtccgtgttggttgcagctggagagacagccactctgcgctgcactgcgacctctctgatccctgtggggcccatccagtggttcagaggagctggaccaggccgggaattaatctacaatcaaaaagaaggccacttcccccgggtaacaactgtttcagacctcacaaagagaaacaacatggacttttccatccgcatcggtaacatcaccccagcagatgccggcacctactactgtgtgaagttccggaaagggagccccgatgacgtggagtttaagtctggagcaggcactgagctgtctgtgcgcgccaaaccctcttga

SEQ ID NO: 7 - protein, 599 aa, H. sapiens
MGWSLILLFLVAVATRVLSQVQLQQPGAELVKPGASVKMSCKASGYTFTSYNMHWVKQTPGRGLEWIGAIYPGNGDTSYNQKFKGKATLTADKSSSTAYMQLSSLTSEDSAVYYCARSTYYGGDWYFNVWGAGTTVTVSAASTKGPSVFPLAPSSKSTSGGTAALGCLVKDYFPEPVTVSWNSGALTSGVHTFPAVLQSSGLYSLSSVVTVPSSSLGTQTYICNVNHKPSNTKVDKKVEPKSCDKTHTCPPCPAPELLGGPSVFLFPPKPKDTLMISRTPEVTCVVVDVSHEDPEVKFNWYVDGVEVHNAKTKPREEQYNSTYRVVSVLTVLHQDWLNGKEYKCKVSNKALPAPIEKTISKAKGQPREPQVYTLPPSRDELTKNQVSLTCLVKGFYPSDIAVEWESNGQPENNYKTTPPVLDSDGSFFLYSKLTVDKSRWQQGNVFSCSVMHEALHNHYTQKSLSLSPGKGGGGSGGGGSEEELQVIQPDKSVLVAAGETATLRCTATSLIPVGPIQWFRGAGPGRELIYNQKEGHFPRVTTVSDLTKRNNMDFSIRIGNITPADAGTYYCVKFRKGSPDDVEFKSGAGTELSVRAKPS

SEQ ID NO: 8 - DNA, 1803 bp, H. sapiens
  CDS (1)...(1803)
atgagggcttggatcttctttctgctctgcctggccgggcgcgccttggccgaggaggagctgcaggtgattcagcctgacaagtccgtgttggttgcagctggagagacagccactctgcgctgcactgcgacctctctgatccctgtggggcccatccagtggttcagaggagctggaccaggccgggaattaatctacaatcaaaaagaaggccacttcccccgggtaacaactgtttcagacctcacaaagagaaacaacatggacttttccatccgcatcggtaacatcaccccagcagatgccggcacctactactgtgtgaagttccggaaagggagccccgatgacgtggagtttaagtctggagcaggcactgagctgtctgtgcgcgccaaaccctctgcgagcaccaagggcccatcggtcttccccctggcaccccaggtacaactgcagcagcctggggctgagctggtgaagcctggggcctcagtgaagatgtcctgcaaggcttctggctacacatttaccagttacaatatgcactgggtaaaacagacacctggtcggggcctggaatggattggagctatttatcccggaaatggtgatacttcctacaatcagaagttcaaaggcaaggccacattgactgcagacaaatcctccagcacagcctacatgcagctcagcagcctgacatctgaggactctgcggtctattactgtgcaagatcgacttactacggcggtgactggtacttcaatgtctggggcgcagggaccacggtcaccgtctctgcagctagcaccaagggcccatcggtcttccccctggcaccctcctccaagagcacctctgggggcacagcggccctgggctgcctggtcaaggactacttccccgaaccggtgacggtgtcgtggaactcaggcgccctgaccagcggcgtgcacaccttcccggctgtcctacagtcctcaggactctactccctcagcagcgtggtgaccgtgccctccagcagcttgggcacccagacctacatctgcaacgtgaatcacaagcccagcaacaccaaggtggacaagaaagttgagcccaaatcttgtgacaaaactcacacatgcccaccgtgcccagcacctgaactcctggggggaccgtcagtctttctcttccccccaaaacccaaggacaccctcatgatctcccggacccctgaggtcacatgcgtggtggtggacgtgagccacgaagaccctgaggtcaagttcaactggtacgtggacggcgtggaggtgcataatgccaagacaaagccgcgggaggagcagtacaacagcacgtaccgtgtggtcagcgtcctcaccgtcctgcaccaggactggctgaatggcaaggagtacaagtgcaaggtctccaacaaagccctcccagcccccatcgagaaaaccatctccaaagccaaagggcagccccgagaaccacaggtgtacaccctgcccccatcccgggatgagctgaccaagaaccaggtcagcctgacctgcctggtcaaaggcttctatcccagcgacatcgccgtggagtgggagagcaatgggcagccggagaacaactacaagaccacgcctcccgtgctggactccgacggctccttcttcctctatagcaagctcaccgtggacaagagcaggtggcagcaggggaacgtcttctcatgctccgtgatgcatgaggctctgcacaaccactacacgcagaagagcctctccctgtctccgggtaaatga

SEQ ID NO: 9 - protein, 600 aa, H. sapiens
MRAWIFFLLCLAGRALAEEELQVIQPDKSVLVAAGETATLRCTATSLIPVGPIQWFRGAGPGRELIYNQKEGHFPRVTTVSDLTKRNNMDFSIRIGNITPADAGTYYCVKFRKGSPDDVEFKSGAGTELSVRAKPSASTKGPSVFPLAPQVQLQQPGAELVKPGASVKMSCKASGYTFTSYNMHWVKQTPGRGLEWIGAIYPGNGDTSYNQKFKGKATLTADKSSSTAYMQLSSLTSEDSAVYYCARSTYYGGDWYFNVWGAGTTVTVSAASTKGPSVFPLAPSSKSTSGGTAALGCLVKDYFPEPVTVSWNSGALTSGVHTFPAVLQSSGLYSLSSVVTVPSSSLGTQTYICNVNHKPSNTKVDKKVEPKSCDKTHTCPPCPAPELLGGPSVFLFPPKPKDTLMISRTPEVTCVVVDVSHEDPEVKFNWYVDGVEVHNAKTKPREEQYNSTYRVVSVLTVLHQDWLNGKEYKCKVSNKALPAPIEKTISKAKGQPREPQVYTLPPSRDELTKNQVSLTCLVKGFYPSDIAVEWESNGQPENNYKTTPPVLDSDGSFFLYSKLTVDKSRWQQGNVFSCSVMHEALHNHYTQKSLSLSPGK

SEQ ID NO: 10 - DNA, 1830 bp, H. sapiens
  CDS (1)...(1830)
atgggttggagcctcatcttgctcttccttgtcgctgttgctacgcgtgtcctgtcccaggtacaactgcagcagcctggggctgagctggtgaagcctggggcctcagtgaagatgtcctgcaaggcttctggctacacatttaccagttacaatatgcactgggtaaaacagacacctggtcggggcctggaatggattggagctatttatcccggaaatggtgatacttcctacaatcagaagttcaaaggcaaggccacattgactgcagacaaatcctccagcacagcctacatgcagctcagcagcctgacatctgaggactctgcggtctattactgtgcaagatcgacttactacggcggtgactggtacttcaatgtctggggcgcagggaccacggtcaccgtctctgcagcgagcaccaagggcccatcggtcttccccctggcaccctcctccaagagcacctctgggggcacagcggccctgggctgcctggtcaaggactacttccccgaaccggtgacggtgtcgtggaactcaggcgccctgaccagcggcgtgcacaccttcccggctgtcctacagtcctcaggactctactccctcagcagcgtggtgaccgtgccctccagcagcttgggcacccagacctacatctgcaacgtgaatcacaagcccagcaacaccaaggtggacaagaaagttgagcccaaatcttgtgacaaaactcacacatgcccaccgtgcccagcacctgaactcctggggggaccgtcagtctttctcttccccccaaaacccaaggacaccctcatgatctcccggacccctgaggtcacatgcgtggtggtggacgtgagccacgaagaccctgaggtcaagttcaactggtacgtggacggcgtggaggtgcataatgccaagacaaagccgcgggaggagcagtacaacagcacgtaccgtgtggtcagcgtcctcaccgtcctgcaccaggactggctgaatggcaaggagtacaagtgcaaggtctccaacaaagccctcccagcccccatcgagaaaaccatctccaaagccaaagggcagccccgagaaccacaggtgtacaccctgcccccatcccgggatgagctgaccaagaaccaggtcagcctgacctgcctggtcaaaggcttctatcccagcgacatcgccgtggagtgggagagcaatgggcagccggagaacaactacaagaccacgcctcccgtgctggactccgacggctccttcttcctctatagcaagctcaccgtggacaagagcaggtggcagcaggggaacgtcttctcatgctccgtgatgcatgaggctctgcacaaccactacacgcagaagagcctctccctgtctccgggtaaaggtggcggtggctcgggcggtggtgggtcgggtggcggcggatctggcggcggtggttctgaggaggagctgcaggtgattcagcctgacaagtccgtgttggttgcagctggagagacagccactctgcgctgcactgcgacctctctgatccctgtggggcccatccagtggttcagaggagctggaccaggccgggaattaatctacaatcaaaaagaaggccacttcccccgggtaacaactgtttcagacctcacaaagagaaacaacatggacttttccatccgcatcggtaacatcaccccagcagatgccggcacctactactgtgtgaagttccggaaagggagccccgatgacgtggagtttaagtctggagcaggcactgagctgtctgtgcgcgccaaaccctcttga

SEQ ID NO: 11 - protein, 609 aa, H. sapiens
MGWSLILLFLVAVATRVLSQVQLQQPGAELVKPGASVKMSCKASGYTFTSYNMHWVKQTPGRGLEWIGAIYPGNGDTSYNQKFKGKATLTADKSSSTAYMQLSSLTSEDSAVYYCARSTYYGGDWYFNVWGAGTTVTVSAASTKGPSVFPLAPSSKSTSGGTAALGCLVKDYFPEPVTVSWNSGALTSGVHTFPAVLQSSGLYSLSSVVTVPSSSLGTQTYICNVNHKPSNTKVDKKVEPKSCDKTHTCPPCPAPELLGGPSVFLFPPKPKDTLMISRTPEVTCVVVDVSHEDPEVKFNWYVDGVEVHNAKTKPREEQYNSTYRVVSVLTVLHQDWLNGKEYKCKVSNKALPAPIEKTISKAKGQPREPQVYTLPPSRDELTKNQVSLTCLVKGFYPSDIAVEWESNGQPENNYKTTPPVLDSDGSFFLYSKLTVDKSRWQQGNVFSCSVMHEALHNHYTQKSLSLSPGKGGGGSGGGGSGGGGSGGGGSEEELQVIQPDKSVLVAAGETATLRCTATSLIPVGPIQWFRGAGPGRELIYNQKEGHFPRVTTVSDLTKRNNMDFSIRIGNITPADAGTYYCVKFRKGSPDDVEFKSGAGTELSVRAKPS

SEQ ID NO: 12 - DNA, 711 bp, H. sapiens
  CDS (1)...(711)
atgagggcttggatcttctttctgctctgcctggccgggcgcgccttggccgatattgtgatgacccagactccactctctctgtccgtcacccctggacagccggcctccatctcctgcaagtcaagtcagagcctcttagatggtgatggaaagacatatttgaattggttgctgcagaagccaggccagtctccacagcgcctaatctatctggtgtctaaactggactctggagtgccagataggttcagtggcagcgggtcagggacagatttcacactgaaaatcagccgggtggaggctgaggatgttggggtttattactgctggcaaggtacacattttcctcggacgttcggtcagggcaccaagctggaaatcaaacgtacggtggcggcgccatctgtcttcatcttcccgccatctgatgagcagttgaaatctggaactgcctctgttgtgtgcctgctgaataacttctatcccagagaggccaaagtacagtggaaggtggataacgccctccaatcgggtaactcccaggagagtgtcacagagcaggacagcaaggacagcacctacagcctcagcagcaccctgacgctgagcaaagcagactacgagaaacacaaagtctacgcctgcgaagtcacccatcagggcctgagctcgcccgtcacaaagagcttcaacaggggagagtgttag

SEQ ID NO: 13 - protein, 236 aa, H. sapiens
MRAWIFFLLCLAGRALADIVMTQTPLSLSVTPGQPASISCKSSQSLLDGDGKTYLNWLLQKPGQSPQRLIYLVSKLDSGVPDRFSGSGSGTDFTLKISRVEAEDVGVYYCWQGTHFPRTFGQGTKLEIKRTVAAPSVFIFPPSDEQLKSGTASVVCLLNNFYPREAKVQWKVDNALQSGNSQESVTEQDSKDSTYSLSSTLTLSKADYEKHKVYACEVTHQGLSSPVTKSFNRGEC

SEQ ID NO: 14 - DNA, 1800 bp, H. sapiens; identical to SEQ ID NO: 6
  CDS (1)...(1800)

SEQ ID NO: 15 - protein, 599 aa, H. sapiens; identical to SEQ ID NO: 7